European Patent Specification EP 3 341 487 B1, published October 1, 2025. Title: Means and methods for production of organic compoundsSAR15413LU. Applicant: Universitaet des Saarlandes. The sequence listing filed with the application follows.

SEQUENCE LISTING (107 sequences)

SEQ ID NO: 1 - protein, 311 aa, P. putida
MTVKISHTADIQAFFNRVAGLDHAEGNPRFKQIILRVLQDTARLIEDLEITEDEFWHAVDYLNRLGGRNEAGLLAAGLGIEHFLDLLQDAKDAEAGLGGGTPRTIEGPLYVAGAPLAQGEARMDDGTDPGVVMFLQGQVFDADGKPLAGATVDLWHANTQGTYSYFDSTQSEFNLRRRIITDAEGRYRARSIVPSGYGCDPQGPTQECLDLLGRHGQRPAHVHFFISAPGHRHLTTQINFAGDKYLWDDFAYATRDGLIGELRFVEDAAAARDRGVQGERFAELSFDFRLQGAKSPDAEARSHRPRALQEG

SEQ ID NO: 2 - DNA, 936 bp, P. putida
atgaccgtgaaaatttcccacactgccgacattcaagccttcttcaaccgggtagctggcctggaccatgccgaaggaaacccgcgcttcaagcagatcattctgcgcgtgctgcaagacaccgcccgcctgatcgaagacctggagattaccgaggacgagttctggcacgccgtcgactacctcaaccgcctgggcggccgtaacgaggcaggcctgctggctgctggcctgggtatcgagcacttcctcgacctgctgcaggatgccaaggatgccgaagccggccttggcggcggcaccccgcgcaccatcgaaggcccgttgtacgttgccggggcgccgctggcccagggcgaagcgcgcatggacgacggcactgacccaggcgtggtgatgttccttcagggccaggtgttcgatgccgacggcaagccgttggccggtgccaccgtcgacctgtggcacgccaatacccagggcacctattcgtacttcgattcgacccagtccgagttcaacctgcgtcggcgtatcatcaccgatgccgagggccgctaccgcgcgcgctcgatcgtgccgtccgggtatggctgcgacccgcagggcccaacccaggaatgcctggacctgctcggccgccacggccagcgcccggcgcacgtgcacttcttcatctcggcaccggggcaccgccacctgaccacgcagatcaactttgctggcgacaagtacctgtgggacgactttgcctatgccacccgcgacgggctgatcggcgaactgcgttttgtcgaggatgcggcggcggcgcgcgaccgcggtgtgcaaggcgagcgctttgccgagctgtcattcgacttccgcttgcagggtgccaagtcgcctgacgccgaggcgcgaagccatcggccgcgggcgttgcaggagggctga

SEQ ID NO: 3 - protein, 304 aa, P. putida
MTVNISHTAEVQQFFEQAAGFCNAAGNPRLKRIVQRLLQDTARLIEDLDISEDEFWHAVDYLNRLGGRGEAGLLVAGLGIEHFLDLLQDAKDQEAGRVGGTPRTIEGPLYVAGAPIAQGEVRMDDGSEEGVATVMFLEGQVLDPHGRPLPGATVDLWHANTRGTYSFFDQSQSAYNLRRRIVTDAQGRYRARSIVPSGYGCDPQGPTQECLDLLGRHGQRPAHVHFFISAPGYRHLTTQINLSGDKYLWDDFAYATRDGLVGEVVFVEGPDGRHAELKFDFQLQQAQGGADEQRSGRPRALQEA

SEQ ID NO: 4 - DNA, 915 bp, P. putida
atgaccgtgaacatttcccatactgccgaggtacagcagttcttcgagcaggccgcaggcttttgtaatgcggccggcaacccacgcctcaaacgcatcgtgcagcgcctgctgcaggataccgcgcggctgatcgaagacctggacatcagcgaagacgagttctggcacgccgtcgattacctcaaccgcctgggcggtcgcggcgaagccgggttgctggtggcggggctgggcatcgaacacttcctcgacctgctgcaggatgccaaggaccaggaggcagggcgcgttggcggcaccccacgcaccatcgaaggcccgttgtacgtggctggcgcaccgattgcccaaggtgaagtgcgcatggacgacggcagcgaggagggcgtggccacggtgatgttcctggaaggccaggtgctggacccgcacggacgcccgctgccgggtgccacggtcgacctgtggcatgccaatacccgtggtacctactcgttcttcgaccaaagccagtcggcgtacaacctgcgtcggcgcatcgttaccgatgcccaggggcgctaccgcgcgcgctccatcgtgccatcgggctatggctgcgacccgcaggggccaacccaggaatgcctggacctgctgggccgtcatggccagcgcccggcgcacgtgcacttctttatctcggccccagggtaccggcacctgaccacgcagataaacctgtcgggggacaagtacctgtgggatgactttgcctatgccacacgggatgggctggtcggggaggtggtgttcgtcgaagggccggatggtcggcatgccgagctgaagttcgacttccagttgcagcaggcccagggcggtgccgatgagcagcgcagcgggcggccgcgagctttgcaggaggcctga

SEQ ID NO: 5 - DNA, 81 bp, artificial
  Promoter sequence
tgttgacaattaatcatcggcatagtatatcggcatagtataatacgacaaggtgaggaactaaaccaggaggaaaaacat

SEQ ID NO: 6 - DNA, 85 bp, artificial
  Promoter sequence
tgttgacaattaatcatcggcatagtatatcggcatagtataatacgacaaggtgaggaactaaaccaaagaggagaaattaagc

SEQ ID NO: 7 - DNA, 500 bp, artificial
  Promoter sequence
ccgcttcacagggaacaccactcaggtggtagaactggaagcggtgtcaaagcagctaagtttcagatttgattgaaaaaatttgaaaaaacgcttgacactaggacggcagacaaatagaatgccggccacatctggagggattcccgagcggtcaaaggggacggactgtaaatccgttgcgagagcttcgaaggttcgaatccttctccctccaccagttttagcgagagccgcaagctccgcgggtatagtttagtggtagaacctcagccttccaagctgatgatgcgggttcgattcccgctacccgctccaagtttgtcggattttgcacaaagtgtttcgctcttgtagctcagttggtagagcacacccttggtaagggtgaggtcagcggttcaagtccgctcaagagctccatataaacaaggcagatatgaaaatatctgcctttgttttatcagtgcaagactatttcttctgcggaggattgtatc

SEQ ID NO: 8 - DNA, 499 bp, artificial
  Promoter sequence
ggtcgagccgcccacgctggccgccctgcgcaccctgctgcaccacccactgctggccggcaaggtggaagatgccagccacttcgccgacgaagaacacctgtacagccagctgctggtggcattgatcgaagccgcgcagaaaaatcctgggctaagctcaatgcagttgatcgcacgttggcatggcaccgaacagggccgcctgctacgcgccctggcggaaaaggaatggcttatcgtggccgacaaccttgaacaacagtttttcgacactataactagcttgtccgcccgccaacgcgagcgcagcctggaacaactgctcaggaaatcacgtcaaagcgaattgaccagcgaggaaaaaacccagctcctcgccctgctgagccgaaatgttcccgcacaaacgccgacctcatctggcgcgtgaggcccatgctcgggtataatcctcggcttgttttttgcccgccaagaccttcagtggatagggtgt

SEQ ID NO: 9 - DNA, 31 bp, artificial
  Promoter sequence
tttacactttatgcttccggctcgtatggtt

SEQ ID NO: 10 - DNA, 500 bp, artificial
  Promoter sequence
aaccagtctttccatatagagcatgtgatggacggtgcctgttgatcagtgcccaaggggtgcttgatcggacacacggatcggggacaacatgaaaaaaaagaagagacatataaaaagcttttttgaagaacttataactcttaagtggataaccttctgtggataacctgcgctggcccatgaattacggggtgtacagagttttacaactttgttctgatcccgtgctgcgcttgttccaatcgtgagcgaaagctgtggatgaaaacacctgttatccacagcggagttatcaacaggctaaggggtggggttgtgcatagccctcatggtcgtttatccacagggcttattcacagaggcgaaaagccgttttggtcgataaatggctgttttgtcgtggttcctaacgtgtccacatgtggataactgaacgctcgaccggtacaatggcggtttgtttttgcctcatccggctttcaaactcaggggatatc

SEQ ID NO: 11 - DNA, 72 bp, artificial
  Promoter sequence
tgttgacaattaatcatcggcatagtatagtacgacaaggtgaggaactaaaccaaagaggagaaattaagc

SEQ ID NO: 12 - DNA, 84 bp, artificial
  Promoter sequence
tgttgacaattaatcatcggcacagtatgctggcatagtacaatacaacaaggtggggaactagaccaaagaggagaaattaag

SEQ ID NO: 13 - DNA, 70 bp, artificial
  Promoter sequence
tgttgacattaatctcggcatagtataatacgacaaggtgaggaactaaaccaaagaggagaaattaagc

SEQ ID NO: 14 - DNA, 72 bp, artificial
  Promoter sequence
tgttgacaattaatcatcggcatagtatagtatgacaaagtgaggaactgagccaaagaggagaaattaagc

SEQ ID NO: 15 - DNA, 70 bp, artificial
  Promoter sequence
tgttgacaattatctcggcatagtataatacgacaaggtgaggaactaaaccaaagaggagaaattaagc

SEQ ID NO: 16 - DNA, 85 bp, artificial
  Promoter sequence
tgttgacaattaatcatcggcatagtatattggcgtagtgtagtacggcaaggtggggaactgagccaaagaggagaaattaagc

SEQ ID NO: 17 - protein, 500 aa, Klebsiella pneumoniae
MTAPIQDLRDAIALLQQHDNQYLETDHPVDPNAELAGVYRHIGAGGTVKRPTRIGPAMMFNNIKGYPHSRILVGMHASRQRAALLLGCEASQLALEVGKAVKKPVAPVVVPASSAPCQEQIFLADDPDFDLRTLLPAPTNTPIDAGPFFCLGLALASDPVDASLTDVTIHRLCVQGRDELSMFLAAGRHIEVFRQKAEAAGKPLPITINMGLDPAIYIGACFEAPTTPFGYNELGVAGALRQRPVELVQGVSVPEKAIARAEIVIEGELLPGVRVREDQHTNSGHAMPEFPGYCGGANPSLPVIKVKAVTMRNNAILQTLVGPGEEHTTLAGLPTEASIWNAVEAAIPGFLQNVYAHTAGGGKFLGILQVKKRQPADEGRQGQAALLALATYSELKNIILVDEDVDIFDSDDILWAMTTRMQGDVSITTIPGIRGHQLDPSQTPEYSPSIRGNGISCKTIFDCTVPWALKSHFERAPFADVDPRPFAPEYFARLEKNQGS

SEQ ID NO: 18 - DNA, 1509 bp, K. pneumoniae
atgaccgcaccgattcaggatctgcgcgacgccatcgcgctgctgcaacagcatgacaatcagtatctcgaaaccgatcatccggttgaccctaacgccgagctggccggtgtttatcgccatatcggcgcgggcggcaccgtgaagcgccccacccgcatcgggccggcgatgatgtttaacaatattaagggttatccacactcgcgcattctggtgggtatgcacgccagccgccagcgggccgcgctgctgctgggctgcgaagcctcgcagctggcccttgaagtgggtaaggcggtgaaaaaaccggtcgcgccggtggtcgtcccggccagcagcgccccctgccaggaacagatctttctggccgacgatccggattttgatttgcgcaccctgcttccggcgcccaccaacacccctatcgacgccggccccttcttctgcctgggcctggcgctggccagcgatcccgtcgacgcctcgctgaccgacgtcaccatccaccgcttgtgcgtccagggccgggatgagctgtcgatgtttcttgccgccggccgccatatcgaagtgtttcgccaaaaggccgaggccgccggcaaaccgctgccgataaccatcaatatgggtctcgatccggccatctatattggcgcctgcttcgaagcccctaccacgccgttcggctataatgagctgggcgtcgccggcgcgctgcgtcaacgtccggtggagctggttcagggcgtcagcgtcccggagaaagccatcgcccgcgccgagatcgttatcgaaggtgagctgttgcctggcgtgcgcgtcagagaggatcagcacaccaatagcggccacgcgatgccggaatttcctggctactgcggcggcgctaatccgtcgctgccggtaatcaaagtcaaagcagtgaccatgcgaaacaatgcgattctgcagaccctggtgggaccgggggaagagcataccaccctcgccggcctgccaacggaagccagtatctggaatgccgtcgaggccgccattccgggctttttacaaaatgtctacgcccacaccgcgggtggcggtaagttcctcgggatcctgcaggtgaaaaaacgtcaacccgccgatgaaggccggcaggggcaggccgcgctgctggcgctggcgacctattccgagctaaaaaatattattctggttgatgaagatgtcgacatctttgacagcgacgatatcctgtgggcgatgaccacccgcatgcagggggacgtcagcattacgacaatccccggcattcgcggtcaccagctggatccgtcccagacgccggaatacagcccgtcgatccgtggaaatggcatcagctgcaagaccatttttgactgcacggtcccctgggcgctgaaatcgcactttgagcgcgcgccgtttgccgacgtcgatccgcgtccgtttgcaccggagtatttcgcccggctggaaaaaaaccagggtagcgcaaaataa

SEQ ID NO: 19 - protein, 197 aa, K. pneumoniae
MKLIIGMTGATGAPLGVALLQALRDMPEVETHLVMSKWAKTTIELETPWTAREVAALADFSHSPADQAATISSGSFRTDGMIVIPCSMKTLAGIRAGYAEGLVGRAADVVLKEGRKLVLVPREMPLSTIHLENMLALSRMGVAMVPPMPAYYNHPETVDDITNHIVTRVLDQFGLDYHKARRWNGLRTAEQFAQEIE

SEQ ID NO: 20 - DNA, 594 bp, K. pneumoniae
atgaaactgattattgggatgacgggggccaccggggcaccgcttggggtggcattgctgcaggcgctgcgcgatatgccggaggtggaaacccatctggtgatgtcgaaatgggccaaaaccaccatcgagctggaaacgccctggacggcgcgcgaagtggccgcgctggcggacttttcccacagcccggcagaccaggccgccaccatctcatccggttcatttcgtaccgacggcatgatcgttattccctgcagtatgaaaacgcttgcaggcattcgcgcgggttatgccgaaggactggtgggccacgcggcggacgtggtgctcaaagaggggcgcaagctggtgttggtcccgcgggaaatgccgctcagcacgatccatctggagaacatgctggcgctgtcccgcatgggcgtggcgatggtcccgccgatgtcagcttactacaaccacccggagacggttgacgatatcaccaatcatatcgtcacccgggtgctggatcagtttggcctcgactatcacaaagcgcgccgctggaacggcttgcgcacggcagaacaatttgcacaggagatcgaataa

SEQ ID NO: 21 - protein, 610 aa, Artificial
  Plasmid pEST1226
MTTQRNDNLEQPGRSVIFDDGLSATDTPNETNVVETEVLIVGSGPAGSSAAMFLSTQGISNIMITKYRWTANTPRAHITNQRTMEILRDAGIEDQVLAEAVPHELMGDTVYCESMAGEEIGRRPTWGTRPDRRADYELASPAMPCDIPQTLLEPIMLKNATMRGTQTQFSTEYLSHTQDDKGVSVQVLNRLTGQEYTIRAKYLIGADGARSKVAADIGGSMNITFKADLSHWRPSALDPVLGLPPRIEYRWPRRWFDRMVRPWNEWLVVWGFDINQEPPKLNDDEAIQIVRNLVGIEDLDVEILGYSLWGNNDQYATHLQKGRVCCAGDAIHKHPPSHGLGSNTSIQDSYNLCWKLACVLKGQAGPELLETYSTERAPIAKQIVTRANGSSSEYKPIFDALGVTDATTNDEFVEKLALRKENSPEGARRRAALRAALDNKDYEFNAQGTEIGQFYDSSAVITDGQKRPAMTEDPMLHHQKSTFPGLRLPHAWLGDAKEKYSTHDIAEGTRFTIFTGITGQAWADAAVRVAERLGIDLKAVVIGEGQPVQDLYGDWLRQREVDEDGVILVRPDKHIGWRAQSMVADPETALFDVLSALLHTKQTGSSHLRV

SEQ ID NO: 22 - DNA, 1833 bp, Artificial
  Plasmid pEST1226
atgactacacagcgtaatgataatcttgagcagccgggccgtagcgtcatttttgatgatgggctgagcgcaactgataccccaaatgagaccaacgtagttgaaactgaggtgttaattgtcggttcaggccctgctggcagctccgcagcaatgttcctgtcgacccagggcattagcaacattatgatcaccaaataccgttggactgcgaataccccccgtgcgcatatcactaaccagcgcaccatggaaattttacgcgacgctggtattgaggatcaggttttagcagaagcagtcccccatgaacttatgggtgacacagtctattgtgagtcaatggccggcgaagaaattggccgccggccaacttggggcacacgacctgaccgccgcgctgactatgagctggcatctccagcgatgccttgcgatatcccgcaaaccttgcttgagcccattatgctcaaaaatgccaccatgcgtggcacgcaaacacagttctccactgagtatttaagccacacccaagacgataagggtgtcagcgtgcaagtactcaaccgtctgaccggtcaagaatataccattcgcgccaaatacctgattggtgctgatggtgcgcgctccaaagtggctgcggatatcggcggctcgatgaatatcacctttaaagcagacttgtcccactggcgcccatcggccctcgatcctgtattgggtcttccgcccaggatcgaatatcggtggcctcggcgctggtttgatcgcatggtgcggccatggaatgaatggctggtggtctggggttttgatatcaatcaagagccacccaagctcaatgacgatgaagctattcaaatcgtgcgtaatctagtgggtatcgaggatcttgatgtggaaatccttggctactcactctggggcaataatgaccagtacgccacgcatctacagaaaggccgcgtatgctgtgccggtgatgcaatccataagcatccgcccagtcacggcctgggttctaatacgtcaatccaagactcctacaacctgtgctggaagttggcctgtgtactcaaagggcaggcggggcctgaactgttagaaacctattccaccgagcgtgcacccatcgccaagcagattgtgacgcgtgccaacggctcgagcagtgaatataagccgatttttgacgctttaggcgttaccgatgcgacaaccaacgatgagtttgtagaaaagcttgccttgcgtaaggaaaattcgcctgaaggtgctcgccgtcgagcagcattgcgtgcggcgctggacaataaggattatgagtttaacgcccaaggcactgaaattggtcagttctacgactcatcagcagtgattactgatggtcaaaaacgcccagcaatgaccgaggatcctatgctacaccaccagaaatcgacctttcctggactacgcctaccccatgcatggctaggtgatgcgaaagagaaatactccacccatgatattgcggagggcactcgcttcacgattttcactggtatcaccggtcaagcttgggctgatgcagcagttcgcgttgctgagcgtttgggcatcgacttgaaggccgtggtgattggtgaagggcagccggtacaagacctctatggcgattggttacgccagcgtgaagtggacgaggacggtgtgatcttggtgcgcccagataaacatattggttggcgtgcccagagtatggtcgcagatccagagactgcattatttgatgtactctcagcgctgctgcataccaagcaaaccggctcttcgcatttaagggtgtag

SEQ ID NO: 23 - protein, 521 aa, P. putida
MSEQNNAVLPKGVTQGEFNKAVQKFRALLGDDNVLVESDQLVPYNKIMMPVENAAHAPSAAVTATTVEQVQGVVKICNEHKIPIWTISTGRNFGYGSAAPVQRGQVILDLKKMNKIIKIDPEMCYALVEPGVTFGQMYDYIQENNLPVMLSFSAPSAIAGPVGNTMDRGVGYTPYGEHFMMQCGMEVVLANGDVYRTGMGGVPGSNTWQIFKWGYGPTLDGMFTQANYGICTKMGFWLMPKPPVFKPFEVIFEDEADIVEIVDALRPLRMSNTIPNSVVIASTLWEAGSAHLTRAQYTTEPGHTPDSVIKQMQKDTGMGAWNLYAALYGTQEQVDVNWKIVTDVFKKLGKGRIVTQEEAGDTQPFKYRAQLMSGVPNLQEFGLYNWRGGGGSMWFAPVSEARGSECKKQAAMAKRVLHKYGLDYVAEFIVAPRDMHHVIDVLYDRTNPEETKRADACFNELLDEFEKEGYAVYRVNTRFQDRVAQSYGPVKRKLEHAIKRAVDPNNILAPGRSGIDLNNDF

SEQ ID NO: 24 - DNA, 1566 bp, P. putida
atgtccgagcaaaacaatgctgtgttgcccaaaggggtaacgcagggcgagttcaacaaggcggtgcagaaattccgcgccttgctgggtgacgataatgtattggtcgaatccgaccagttggtgccttacaacaagatcatgatgccggtcgagaatgcggctcatgccccctcggccgccgtcaccgcgaccaccgtcgagcaggtgcagggtgtagtcaagatctgtaacgaacacaaaattccgatctggaccatctccactgggcgcaacttcggttacgggtccgccgcgccggtgcagcgcggtcaggtaatccttgacctgaagaagatgaacaagatcatcaagatcgacccggaaatgtgctatgcgctggtcgagccgggggttaccttcggtcagatgtatgactacatccaggaaaacaacctgccggtgatgctgtcgttctcggcaccctcggcgattgccggcccggtcggcaataccatggaccgaggcgtgggctacaccccctacggcgaacacttcatgatgcagtgcggcatggaagtggtgctggccaacggtgacgtttaccgcaccggcatgggtggcgtgcctggcagcaacacctggcagattttcaaatggggctatggtccgaccctggatggcatgttcactcaggccaactatggcatttgcaccaagatgggcttctggctgatgcccaagccgcccgtgttcaagccgttcgaagtgatcttcgaggacgaggcggacatcgtcgagatcgtcgatgcactgcgcccgctgcgcatgagcaacaccatccccaactcggtggtaatcgccagcaccttgtgggaagccggcagtgcgcacctgacccgcgcccagtacaccaccgagccgggccacacgccggatagcgtgatcaagcagatgcagaaagacaccggcatgggtgcctggaacctctacgctgcgctgtacggtacccaggaacaggtcgacgtaaactggaagatcgtaactgacgtcttcaagaaacttggcaagggccgtatcgtcacccaggaagaggcgggtgacacccagccgttcaaataccgtgcccagctgatgtccggcgtgcccaacctgcaggaattcggcctgtacaactggcgtgggggcggtggctccatgtggttcgcgccggtcagcgaggcgcgtggcagcgagtgcaagaagcaggcggccatggccaagcgcgttctgcacaagtacggcctggattatgtggccgagttcatcgtggcgccgcgcgacatgcaccacgtcatcgacgtgctctacgaccgcaccaatcctgaggaaaccaagcgcgccgacgcctgcttcaatgagctgctggatgagttcgagaaggaaggctatgcggtgtatcgggtgaacacccgcttccaggatcgcgtggcgcagagctatggcccggtcaagcgcaagctggagcatgccatcaagcgtgcggtggacccgaacaacatcctcgctccgggccgctcgggcatcgacctcaataacgatttctga

SEQ ID NO: 25 - protein, 113 aa, P. putida
MTFPFSGAAVKRMLVTGVVLPFGLLVAAGQAQADSQWGSGKNLYDKVCGHCHKPEVGVGPVLEGRGLPEAYIKDIVRNGFRAMPAFPASYVDDESLTQVAEYLSSLPAPAAQP

SEQ ID NO: 26 - DNA, 342 bp, P. putida
atgacatttccctttagcggcgcagctgtgaaacggatgctcgtgactggagttgtgcttccctttggtctgctggtcgcagcgggacaggcgcaggccgacagccagtggggcagtggcaagaacctgtatgacaaggtttgtggccattgccacaagcccgaagtcggggtagggccggttcttgagggtcgcggcctgccggaagcctacatcaaggacattgtgcgcaacggcttccgtgccatgccggcattcccggcgtcttatgttgatgacgaatcccttactcaggtggctgaatacctgtcgagcctgccggccccagcggctcagccttga

SEQ ID NO: 27 - protein, 373 aa, Pseudomonas putida
MTSVLIEHIDAIIVDLPTIRPHKLAMHTMQQQTLVVLRLRCSDGVEGIGEATTIGGLAYGYESPEGIKANIDAYLAPALIGLPADNINAAMLKLDKLAKGNTFAKSGIESALLDAQGKRLGLPVSELLGGRVRDSLEVAWTLASGDTARDIAEAQHMLDIRRHRVFKLKIGANPVAQDLKHVVAIKRELGDSASVRVDVNQYWDESQAIRACQVLGDNGIDLIEQPISRINRAGQVRLNQRSPAPIMADESIESVEDAFSLAADGAASIFALKIAKNGGPRAVLRTAQIAEAAGIALYGGTMLEGSIGTLASAHAFLTLRQLTWGTELFGPLLLTEEIVNEPPQYRDFQLHIPHTPGLGLTLDEQRLARFARR

SEQ ID NO: 28 - DNA, 1122 bp, P. putida
atgacaagcgtgctgattgaacacatagatgcaattatcgtcgatctcccgaccattcgcccgcacaagctggcgatgcacaccatgcagcagcagaccctggtggtattgcgactgcgctgcagcgatggcgtggaaggcatcggtgaagccaccaccatcggtggcctggcgtatggctacgaaagccccgaagggatcaaggccaacatcgacgcgtacctcgccccagcgttgattggcctgccggcagacaacatcaatgccgccatgctcaagctggacaagctggccaagggcaacaccttcgccaagtccggcatcgaaagcgccttgctcgacgcccagggcaaacgcctgggcctgccggtcagcgaactgctgggtggccgcgtgcgtgacagcctggaagtggcctggaccctggccagcggcgacaccgcccgcgacatcgccgaagcacagcacatgctggacattcgccggcaccgcgtgttcaagctgaaaatcggcgccaacccggtggcgcaggacctcaagcacgtggtcgcgatcaagcgcgagctgggtgacagcgccagcgtgcgggtcgacgtcaaccagtactgggacgagtcccaggccatccgcgcctgccaggtattgggcgacaacggcatcgacctgatcgagcagccgatttcgcgcatcaaccgcgctggccaggtgcgcctgaaccagcgcagtccggctccgatcatggccgatgagtcgatcgaaagcgtcgaggacgccttcagcctggccgccgacggcgccgccagcatcttcgccctgaaaatcgccaagaatggtggcccgcgcgcggttctgcgcactgcacagatcgccgaggccgctggcatcgccttgtacggcggcaccatgctcgaaggttcgatcggcaccctggcttcggctcatgcattcctcaccctgcgccagctcacctggggtacagagctgttcgggccgctgctgctgaccgaggagatcgtcaacgagccgccgcaataccgcgacttccagctgcacatcccccacaccccaggcctgggcctgacgttggacgaacagcgcctggcgcgcttcgcccgtcgctga

SEQ ID NO: 29 - protein, 96 aa, P. putida
MLFHVKMTVKLPVDMDPAKAAQLKADEKELAQRLQREGIWRHLWRIAGHYANYSVFDVPSVEALHDTLMQLPLFPYMDIEVDGLCRHPSSIHSDDR

SEQ ID NO: 30 - DNA, 291 bp, P. putida
atgttgttccacgtgaagatgaccgtgaagctgccggtcgacatggacccggccaaggccgcccagctcaaggccgacgaaaaggaactggcccagcgcctgcagcgcgaaggcatctggcgtcacctgtggcgcattgccgggcattacgccaactacagcgtgttcgatgtgcccagcgtcgaggcattgcatgacacgctgatgcagctgccgctgttcccgtacatggatatcgaggtcgacggcctgtgtcggcatccctcgtctattcacagcgacgatcgctga

SEQ ID NO: 31 - protein, 450 aa, P. putida
MSNQLFDAYFTAPAMREIFSDRGRLQGMLDFEAALARAEASAGLVPHSAVAAIEAACQAERYDVGALANAIATAGNSAIPLVKALGKVIATGVPEAERYVHLGATSQDAMDTGLVLQLRDALDLIEADLGKLADTLSQQALKHADTPLVGRTWLQHATPVTLGMKLAGVLGALTRHRQRLQELRPRLLVLQFGGASGSLAALGSKAMPVAEALAEQLKLTLPEQPWHTQRDRLVEFASVLGLVAGSLGKFGRDISLLMQTEAGEVFEPSAPGKGGSSTMPHKRNPVGAAVLIGAATRVPGLLSTLFAAMPQEHERSLGLWHAEWETLPDICCLVSGALRQAQVIAEGMEVDAARMRRNLDLTQGLVLAEAVSIVLAQRLGRDRAHHLLEQCCQRAVAEQRHLRAVLGDEPQVSAELSGEELDRLLDPAHYLGQARVWVARAVSEHQRFTA

SEQ ID NO: 32 - DNA, 1353 bp, P. putida
atgagcaaccaactgttcgacgcctatttcaccgcgccggccatgcgcgagattttctccgaccgaggccgcctgcagggcatgctggatttcgaagccgcgcttgcccgagccgaagcctctgccggtttggtcccgcacagcgcggtagcggccatcgaggcggcatgccaggccgagcgctatgacgttggcgcgctggccaatgccatcgccaccgcgggcaactcggccattccgctggtgaaagcgttgggcaaggtgatcgccaccggcgtgccagaggctgagcgctatgtgcaccttggggccaccagccaggatgcgatggataccggtctggttctgcagctgcgcgatgccctcgatttgatcgaggccgacctcggcaagctggccgataccctgtcgcagcaggccttgaagcacgccgatacgcccttggtgggtcgtacctggttgcaacacgccaccccggtgaccctgggcatgaaactggccggtgtactgggtgctttgacccgccaccgtcagcgcctgcaggaactgcgcccgcgccttctggtcctgcagttcggcggtgcctcgggcagcctggcggcgctgggcagcaaggcgatgccggtggccgaagcgctggccgaacagctcaagctgaccctgcccgagcagccctggcacacccagcgcgaccgcctggtggagtttgcctcggtattgggcctggttgccggcagcctgggcaagttcggccgtgatatcagcttgctgatgcaaaccgaggcgggggaggtgtttgagccttctgcgccgggcaagggtggttcttcgaccatgccacacaagcgcaacccggtgggtgccgccgtgttgatcggtgccgcgacccgcgtgccgggcctgctgtcgacgctgttcgcagccatgcctcaggagcacgaacgcagcctgggcctatggcatgccgagtgggaaaccctgccggatatctgctgcctggtctctggcgccctgcgccaggctcaagtgattgccgagggcatggaggtggatgccgcgcgcatgcgccgtaacctcgacctgacccaaggcctggtgctggccgaagcggtgagcatcgtcctcgcccagcgtctgggtcgcgaccgtgcccaccacctgctggaacaatgctgccaacgcgcggtggccgaacagcggcacctgcgtgccgtgctgggtgacgagccgcaggtcagcgccgagctgtctggcgaagaactcgatcgcctgctcgaccctgcccattacctgggccaggcccgcgtctgggtggcgcgcgccgtgtccgaacatcaacgtttcactgcctga

SEQ ID NO: 33 - DNA, 1509 bp, Artificial
  aroY codon optimized
atgaccgcgccgatccaggacctgcgcgatgcgatcgcgctgttgcagcagcatgacaaccagtacctggaaaccgatcatccggtcgatcccaacgccgaactggcgggcgtctaccgccacatcggtgccggcgggaccgtgaagcgtcccacccggatcggtcccgccatgatgttcaacaacatcaagggctatccccattcccgcattctggtcggcatgcacgcgagtcgccaacgggccgctctgctgttgggctgcgaagccagccaactggcactggaggtggggaaagcggtcaagaagccagtagccccggtagtggtgcccgccagtagcgcaccttgtcaggaacagatcttcctggcggatgacccggacttcgacctgcgcaccttgctgcctgccccgacgaatacgccgatcgatgctggcccgttcttctgcctgggcctcgccctcgcgagcgatccagtggacgcaagcctcaccgatgtcaccattcaccgcctgtgtgtgcaggggcgcgacgaactgagcatgttcctcgcagctggtcgccacatcgaagtgttccgccaaaaggccgaggccgcgggcaaacccctgcccattaccatcaacatgggcctggacccggccatctacatcggcgcttgctttgaggctccgaccactccgttcggctacaacgaactcggcgtagccggcgccttgcgccaacgcccagtagagctggttcagggtgtgtcggtgcccgagaaagcgattgcccgtgccgagatcgtcatcgaaggcgaactgctccctggcgttcgcgtccgcgaggaccagcacaccaattcgggccatgcgatgccagagtttccaggctattgcggtggcgccaatccgagcttgccggtgatcaaggtcaaagccgtgaccatgcggaacaacgcgatcctgcagaccctggtgggccctggggaggagcacaccactctggcggggctgccgaccgaagccagcatctggaatgcggtggaagctgccatccccggcttcctgcagaacgtctacgcccacactgcgggtggcggcaagttcctggggattctgcaggttaagaagcggcaaccggccgacgaaggccgccagggtcaggccgccttgctggcactggccacctactccgaactgaagaacatcatcctggtggacgaggatgtggacatcttcgacagcgacgacatcctgtgggccatgacgacccgcatgcagggtgacgtgtcgatcaccaccattccgggcattcgcggtcaccagctggatcctagccagacgcccgagtattcgccgagcatccgcggcaacggcatctcctgcaagacgatcttcgactgcaccgtgccgtgggccctgaagagccactttgagcgtgcaccgtttgccgacgtcgacccgcgtccgttcgccccagagtacttcgcacgtttggagaagaaccagggctcggccaaatga

SEQ ID NO: 34 - DNA, 594 bp, Artificial
  kpdB codon optimized
atgaagctgatcatcgggatgaccggtgccactggcgctcccttgggtgttgccctcctgcaggcactgcgcgacatgccagaggtcgaaacccacctggtgatgtccaagtgggccaagacgaccattgagctggaaaccccgtggacggctcgcgaagtggcagcgttggcggacttcagccacagtccagccgatcaagcggccaccatctcgagcgggagctttcggaccgatggcatgatcgtcatcccgtgctcgatgaaaaccctggccggtattcgcgcaggctatgccgaaggcctggtcggccatgccgccgatgtggtcctgaaggagggccgtaagctcgtgctggtgcctcgcgagatgcccctgtccacgatccacctggagaacatgctggccttgagccgcatgggcgtagccatggttccgccgatgagcgcctactacaaccatccggaaaccgtggacgacatcaccaaccacatcgtgacccgggtactcgaccagttcggcctggactaccacaaagcgcgccgctggaatggcctgcgtaccgcggaacagttcgcgcaggagatcgagtga

SEQ ID NO: 35 - DNA, 2193 bp, Artificial
  Artificial construct
tgttgacaattaatcatcggcatagtatagtacgacaaggtgaggaactaaaccaaagaggagaaattaagcatgaccgcaccgattcaggatctgcgcgacgccatcgcgctgctgcaacagcatgacaatcagtatctcgaaaccgatcatccggttgaccctaacgccgagctggccggtgtttatcgccatatcggcgcgggcggcaccgtgaagcgccccacccgcatcgggccggcgatgatgtttaacaatattaagggttatccacactcgcgcattctggtgggtatgcacgccagccgccagcgggccgcgctgctgctgggctgcgaagcctcgcagctggcccttgaagtgggtaaggcggtgaaaaaaccggtcgcgccggtggtcgtcccggccagcagcgccccctgccaggaacagatctttctggccgacgatccggattttgatttgcgcaccctgcttccggcgcccaccaacacccctatcgacgccggccccttcttctgcctgggcctggcgctggccagcgatcccgtcgacgcctcgctgaccgacgtcaccatccaccgcttgtgcgtccagggccgggatgagctgtcgatgtttcttgccgccggccgccatatcgaagtgtttcgccaaaaggccgaggccgccggcaaaccgctgccgataaccatcaatatgggtctcgatccggccatctatattggcgcctgcttcgaagcccctaccacgccgttcggctataatgagctgggcgtcgccggcgcgctgcgtcaacgtccggtggagctggttcagggcgtcagcgtcccggagaaagccatcgcccgcgccgagatcgttatcgaaggtgagctgttgcctggcgtgcgcgtcagagaggatcagcacaccaatagcggccacgcgatgccggaatttcctggctactgcggcggcgctaatccgtcgctgccggtaatcaaagtcaaagcagtgaccatgcgaaacaatgcgattctgcagaccctggtgggaccgggggaagagcataccaccctcgccggcctgccaacggaagccagtatctggaatgccgtcgaggccgccattccgggctttttacaaaatgtctacgcccacaccgcgggtggcggtaagttcctcgggatcctgcaggtgaaaaaacgtcaacccgccgatgaaggccggcaggggcaggccgcgctgctggcgctggcgacctattccgagctaaaaaatattattctggttgatgaagatgtcgacatctttgacagcgacgatatcctgtgggcgatgaccacccgcatgcagggggacgtcagcattacgacaatccccggcattcgcggtcaccagctggatccgtcccagacgccggaatacagcccgtcgatccgtggaaatggcatcagctgcaagaccatttttgactgcacggtcccctgggcgctgaaatcgcactttgagcgcgcgccgtttgccgacgtcgatccgcgtccgtttgcaccggagtatttcgcccggctggaaaaaaaccagggtagcgcaaaataaaaagaggagaaattaagcatgaagctgatcatcgggatgaccggtgccactggcgctcccttgggtgttgccctcctgcaggcactgcgcgacatgccagaggtcgaaacccacctggtgatgtccaagtgggccaagacgaccattgagctggaaaccccgtggacggctcgcgaagtggcagcgttggcggacttcagccacagtccagccgatcaagcggccaccatctcgagcgggagctttcggaccgatggcatgatcgtcatcccgtgctcgatgaaaaccctggccggtattcgcgcaggctatgccgaaggcctggtcggccatgccgccgatgtggtcctgaaggagggccgtaagctcgtgctggtgcctcgcgagatgcccctgtccacgatccacctggagaacatgctggccttgagccgcatgggcgtagccatggttccgccgatgagcgcctactacaaccatccggaaaccgtggacgacatcaccaaccacatcgtgacccgggtactcgaccagttcggcctggactaccacaaagcgcgccgctggaatggcctgcgtaccgcggaacagttcgcgcaggagatcgagtga

SEQ ID NO: 36 - DNA, 3947 bp, Artificial
  artificial construct
ttgttgacaattaatcatcggcatagtatatcggcatagtataatacgacaaggtgaggaactaaacccctaggttaaagaggagaaattaagcatgtccgagcaaaacaatgctgtgttgcccaaaggggtaacgcagggcgagttcaacaaggcggtgcagaaattccgcgccttgctgggtgacgataatgtattggtcgaatccgaccagttggtgccttacaacaagatcatgatgccggtcgagaatgcggctcatgccccctcggccgccgtcaccgcgaccaccgtcgagcaggtgcagggtgtagtcaagatctgtaacgaacacaaaattccgatctggaccatctccactgggcgcaacttcggttacgggtccgccgcgccggtgcagcgcggtcaggtaatccttgacctgaagaagatgaacaagatcatcaagatcgacccggaaatgtgctatgcgctggtcgagccgggggttaccttcggtcagatgtatgactacatccaggaaaacaacctgccggtgatgctgtcgttctcggcaccctcggcgattgccggcccggtcggcaataccatggaccgaggcgtgggctacaccccctacggcgaacacttcatgatgcagtgcggcatggaagtggtgctggccaacggtgacgtttaccgcaccggcatgggtggcgtgcctggcagcaacacctggcagattttcaaatggggctatggtccgaccctggatggcatgttcactcaggccaactatggcatttgcaccaagatgggcttctggctgatgcccaagccgcccgtgttcaagccgttcgaagtgatcttcgaggacgaggcggacatcgtcgagatcgtcgatgcactgcgcccgctgcgcatgagcaacaccatccccaactcggtggtaatcgccagcaccttgtgggaagccggcagtgcgcacctgacccgcgcccagtacaccaccgagccgggccacacgccggatagcgtgatcaagcagatgcagaaagacaccggcatgggtgcctggaacctctacgctgcgctgtacggtacccaggaacaggtcgacgtaaactggaagatcgtaactgacgtcttcaagaaacttggcaagggccgtatcgtcacccaggaagaggcgggtgacacccagccgttcaaataccgtgcccagctgatgtccggcgtgcccaacctgcaggaattcggcctgtacaactggcgtgggggcggtggctccatgtggttcgcgccggtcagcgaggcgcgtggcagcgagtgcaagaagcaggcggccatggccaagcgcgttctgcacaagtacggcctggattatgtggccgagttcatcgtggcgccgcgcgacatgcaccacgtcatcgacgtgctctacgaccgcaccaatcctgaggaaaccaagcgcgccgacgcctgcttcaatgagctgctggatgagttcgagaaggaaggctatgcggtgtatcgggtgaacacccgcttccaggatcgcgtggcgcagagctatggcccggtcaagcgcaagctggagcatgccatcaagcgtgcggtggacccgaacaacatcctcgctccgggccgctcgggcatcgacctcaataacgatttctgaaaagaggagaaattaagcatgacatttccctttagcggcgcagctgtgaaacggatgctcgtgactggagttgtgcttccctttggtctgctggtcgcagcgggacaggcgcaggccgacagccagtggggcagtggcaagaacctgtatgacaaggtttgtggccattgccacaagcccgaagtcggggtagggccggttcttgagggtcgcggcctgccggaagcctacatcaaggacattgtgcgcaacggcttccgtgccatgccggcattcccggcgtcttatgttgatgacgaatcccttactcaggtggctgaatacctgtcgagcctgccggccccagcggctcagccttgattgttgacaattaatcatcggcatagtatatcggcatagtataatacgacaaggtgaggaactaaacccctaggttaaagaggagaaattaagcatgactacacagcgtaatgataatcttgagcagccgggccgtagcgtcatttttgatgatgggctgagcgcaactgataccccaaatgagaccaacgtagttgaaactgaggtgttaattgtcggttcaggccctgctggcagctccgcagcaatgttcctgtcgacccagggcattagcaacattatgatcaccaaataccgttggactgcgaataccccccgtgcgcatatcactaaccagcgcaccatggaaattttacgcgacgctggtattgaggatcaggttttagcagaagcagtcccccatgaacttatgggtgacacagtctattgtgagtcaatggccggcgaagaaattggccgccggccaacttggggcacacgacctgaccgccgcgctgactatgagctggcatctccagcgatgccttgcgatatcccgcaaaccttgcttgagcccattatgctcaaaaatgccaccatgcgtggcacgcaaacacagttctccactgagtatttaagccacacccaagacgataagggtgtcagcgtgcaagtactcaaccgtctgaccggtcaagaatataccattcgcgccaaatacctgattggtgctgatggtgcgcgctccaaagtggctgcggatatcggcggctcgatgaatatcacctttaaagcagacttgtcccactggcgcccatcggccctcgatcctgtattgggtcttccgcccaggatcgaatatcggtggcctcggcgctggtttgatcgcatggtgcggccatggaatgaatggctggtggtctggggttttgatatcaatcaagagccacccaagctcaatgacgatgaagctattcaaatcgtgcgtaatctagtgggtatcgaggatcttgatgtggaaatccttggctactcactctggggcaataatgaccagtacgccacgcatctacagaaaggccgcgtatgctgtgccggtgatgcaatccataagcatccgcccagtcacggcctgggttctaatacgtcaatccaagactcctacaacctgtgctggaagttggcctgtgtactcaaagggcaggcggggcctgaactgttagaaacctattccaccgagcgtgcacccatcgccaagcagattgtgacgcgtgccaacggctcgagcagtgaatataagccgatttttgacgctttaggcgttaccgatgcgacaaccaacgatgagtttgtagaaaagcttgccttgcgtaaggaaaattcgcctgaaggtgctcgccgtcgagcagcattgcgtgcggcgctggacaataaggattatgagtttaacgcccaaggcactgaaattggtcagttctacgactcatcagcagtgattactgatggtcaaaaacgcccagcaatgaccgaggatcctatgctacaccaccagaaatcgacctttcctggactacgcctaccccatgcatggctaggtgatgcgaaagagaaatactccacccatgatattgcggagggcactcgcttcacgattttcactggtatcaccggtcaagcttgggctgatgcagcagttcgcgttgctgagcgtttgggcatcgacttgaaggccgtggtgattggtgaagggcagccggtacaagacctctatggcgattggttacgccagcgtgaagtggacgaggacggtgtgatcttggtgcgcccagataaacatattggttggcgtgcccagagtatggtcgcagatccagagactgcattatttgatgtactctcagcgctgctgcataccaagcaaaccggctcttcgcatttaagggtgtag

SEQ ID NO: 37 - DNA, 23 bp, artificial
  primer
ccattcaggctgcgcaactgttg

SEQ ID NO: 38 - DNA, 22 bp, artificial
  primer
ctttacactttatgcttccggc

SEQ ID NO: 39 - DNA, 20 bp, artificial
  primer
ggacgcttcgctgaaaacta

SEQ ID NO: 40 - DNA, 20 bp, artificial
  primer
aacgtcgtgactgggaaaac

SEQ ID NO: 41 - DNA, 24 bp, artificial
  primer
ggcacatcgaacacgctgtagttg

SEQ ID NO: 42 - DNA, 24 bp, artificial
  primer
cctccagggtatggtgggagattc

SEQ ID NO: 43 - DNA, 34 bp, artificial
  primer
tgaacgcttcgccagccaactaccttcgccagcc

SEQ ID NO: 44 - DNA, 28 bp, artificial
  primer
gctcgatacccaggccagcaggccagca

SEQ ID NO: 45 - DNA, 28 bp, artificial
  primer
catatgtgttgccaggtcccgtcaggtc

SEQ ID NO: 46 - DNA, 33 bp, artificial
  primer
aaaaacatatgcagctcaaggccgacgaaaagg

SEQ ID NO: 47 - DNA, 40 bp, artificial
  primer
tgaattcgagctcggtaccctgggcgatgtgcagcagctc

SEQ ID NO: 48 - DNA, 41 bp, artificial
  primer
cgatgattaattgtcaacaacgtgcttacctcgtattgttc

SEQ ID NO: 49 - DNA, 42 bp, artificial
  primer
ttaaagaggagaaattaagcatgaccgtgaaaatttcccaca

SEQ ID NO: 50 - DNA, 41 bp, artificial
  primer
gtcgactctagaggatcccctcgaagtacgaataggtgccc

SEQ ID NO: 51 - DNA, 51 bp, artificial
  primer
gcctgacaagaacaatacgaggtaagcacgttgttgacaattaatcatcgg

SEQ ID NO: 52 - DNA, 57 bp, artificial
  primer
gtcggcagtgtgggaaattttcacggtcatgcttaatttctcctctttaacctaggg

SEQ ID NO: 53 - DNA, 4389 bp, artificial
  pEMG-deltacatB catC
  misc_feature (3555)..(3555): n is a, c, g, or t
gccggcgtcccggaaaacgattccgaagcccaacctttcatagaaggcggcggtggaatcgaaatctcgtgatggcaggttgggcgtcgcttggtcggtcatttcgaaccccagagtcccgctcagaagaactcgtcaagaaggcgatagaaggcgatgcgctgcgaatcgggagcggcgataccgtaaagcacgaggaagcggtcagcccattcgccgccaagctcttcagcaatatcacgggtagccaacgctatgtcctgatagcggtccgccacacccagccggccacagtcgatgaatccagaaaagcggccattttccaccatgatattcggcaagcaggcatcgccatgggtcacgacgagatcctcgccgtcgggcatgcgcgccttgagcctggcgaacagttcggctggcgcgagcccctgatgctcttcgtccagatcatcctgatcgacaagaccggcttccatccgagtacgtgctcgctcgatgcgatgtttcgcttggtggtcgaatgggcaggtagccggatcaagcgtatgcagccgccgcattgcatcagccatgatggatactttctcggcaggagcaaggtgagatgacaggagatcctgccccggcacttcgcccaatagcagccagtcccttcccgcttcagtgacaacgtcgagcacagctgcgcaaggaacgcccgtcgtggccagccacgatagccgcgctgcctcgtcctgcagttcattcagggcaccggacaggtcggtcttgacaaaaagaaccgggcgcccctgcgctgacagccggaacacggcggcatcagagcagccgattgtctgttgtgcccagtcatagccgaatagcctctccacccaagcggccggagaacctgcgtgcaatccatcttgttcaatcatgcgaaacgatcctcatcctgtctcttgatcagatcttgatcccctgcgccatcagatccttggcggcaagaaagccatccagtttactttgcagggcttcccaaccttaccagagggcgccccagctggcaattccggttcgcttgctgtccataaaaccgcccagtctagctatcgccatgtaagcccactgcaagctacctgctttctctttgcgcttgcgttttcccttgtccagatagcccagtagctgacattcatccggggtcagcaccgtttctgcggactggctttctacgtgttccgcttcctttagcagcccttgcgccctgagtgcttgcggcagcgtgaagctaattcccatgtcagccgttaagtgttcctgtgtcactcaaaattgctttgagaggctctaagggcttctcagtgcgttacatccctggcttgttgtccacaaccgttaaaccttaaaagctttaaaagccttatatattcttttttttcttataaaacttaaaaccttagaggctatttaagttgctgatttatattaattttattgttcaaacatgagagcttagtacgtgaaacatgagagcttagtacgttagccatgagagcttagtacgttagccatgagggtttagttcgttaaacatgagagcttagtacgttaaacatgagagcttagtacgtgaaacatgagagcttagtacgtactatcaacaggttgaactgctgatcttcagatcctctacgccggacgcatcgtggccgttttccgctgcataaccctgcttcggggtcattatagcgattttttcggtatatccatcctttttcgcacgatatacaggattttgccaaagggttcgtgtagactttccttggtgtatccaacggcgtcagccgggcaggataggtgaagtaggcccacccgcgagcgggtgttccttcttcactgtcccttattcgcacctggcggtgctcaacgggaatcctgctctgcgaggctggccggctaccgccggcgtaacagatgagggcaagcggatggctgatgaaaccaagccaaccaggaagggcagcccacctatcaaggtgtactgccttccagacgaacgaagagcgattgaggaaaaggcggcggcggccggcatgagcctgtcggcctacctgctggccgtcggccagggctacaaaatcacgggcgtcgtggactatgagcacgtccgcgagctggcccgcatcaatggcgacctgggccgcctgggcggcctgctgaaactctggctcaccgacgacccgcgcacggcgcggttcggtgatgccacgatcctcgccctgctggcgaagatcgaagagaagcaggacgagcttggcaaggtcatgatgggcgtggtccgcccgagggcagagccatgacttttttagccgctaaaacggccggggggtgcgcgtgattgccaagcacgtccccatgcgctccatcaagaagagcgacttcgcggagctggtgaagtacatcaccgacgagcaaggcaagaccgaccaaagcggccatcgtgcctccccactcctgcagttcgggggcatggatgcgcggatagccgctgctggtttcctggatgccgacggatttgcactgccggtagaactccgcgaggtcgtccagcctcaggcagcagctgaaccaactcgcgaggggatcgagccccattcgccattcaggctgcgcaactgttgggaagggcgatcggtgcgggcctcttcgctattacgccagctggcgaaagggggatgtgctgcaaggcgattaagttgggtaacgccagggttttcccagtcacgacgttgtaaaacgacggccagtatagggataacagggtaatctgaattcgagctcggtaccctgaacgcttcgccagccaactgggccagactgagcgggctgcccgccagggggtggcccttgggcagcacggccaccagcgggtcctcgcacagcacctgctggtgaatcaccgggtcgtcgatgcgaatgcgcccgaagccaatgtcgatacgcccgcttttcagcgcctccacctgttgcaaggtggtcatttcgttcaggcccagttccagctcgctgtcctggcgcagctcgcggatcagctccggcagcacggtgtacagggtagagggcgcaaagccgatgcccagccactggcgctggccctggccgatgcggcgggtgttgtcgctgatgttctgcaactgctgcagcacggtgcaggtctgttcgtagaagaagcggccggcctcggtcagccgcagcggacgttcgcgcaccaccagcagggtcccgagctggtcctccagctggctgatctgccggctcaggggtggctgggcgatgtgcagcagctcggcggcgcgggtgaagttcagggtctcggccaagactttgaagtaacgcaggtggcgcagctccatcagacctccagggtatggtgggagattcatttgatattggacggtcgtcagggtctcgcgcaatccttcagcaatcaagtaaacgcatcactcgggcctgcaactgaaagcccgacctgacgggacctggcaacacatatgcagctcaaggccgacgaanaggaactggcccagcgcctgcagcgcgaaggcatctggcgtcacctgtggcgcattgccgggcattacgccaactacagcgtgttcgatgtgcccagcgtcgaggcattgcatgacacgctgatgcagctgccgctgttcccgtacatggatatcgaggtcgacggcctgtgtcggcatccctcgtctattcacagcgacgatcgctgattcgcacctgtatgcctgacaagaacaatacgaggtaagcacgatgaccgtgaaaatttcccacactgccgacattcaagccttcttcaaccgggtagctggcctggaccatgccgaaggaaacccgcgcttcaagcagatcattctgcgcgtgctgcaagacaccgcccgcctgatcgaagacctggagattaccgaggacgagttctggcacgccgtcgactacctcaaccgcctgggcggccgtaacgaggcaggcctgctggctgctggcctgggtatcgagcggggatcctctagagtcgacctgcaggcatgcaagcttctagggataacagggtaatccggcgtaatcatggtcatagctgtttcctgtgtgaaattgttatccgctcacaattccacacaacatacgagccggaagcataaagtgtaaagcctggggtgcctaatgagtgagctaactcacattaattgcgttgcgctcactgcccgctttccagtcgggaaacctgtcgtgccagctgcattaatgaatcggccaacgcgcggggagaggcggtttgcgtattggggggtgggcgaagaactccagcatgagatccccgcgctggaggatcatcca

SEQ ID NO: 54 - DNA, 4168 bp, artificial
  pEMG-deltapcaB
acaccgcgggcatgaccgccaagaacgccagctacgtgatgaccggggcgttgttcctgttcatggtggtgcagccgttcttcggcatgctgtccgaccgtatcggccggcgcaattcgatgctgctgttcggcggcctcggtaccctgtgcaccgtgccgctgctgatggcgctgaaaaccgtgaccagcccgatcatggccttcgtgctgatcagcctggccctgtgtatcgtgagtttctacacctcgatcagcggtctggtgaaggccgagatgttcccgccgcaggtgcgtgcactgggtgttggcctggcctacgcggtggccaacgcagcattcggcggttcggccgagtatgtggccctgggcctgaaaaccctggggatggaaaacactttctattggtacgtgacggcgatgatggcgattgccttcctgttcagcctgcgcctgccgaagcaggcggcgtacctgcaccatgatgattaaggacgctgcaggagaccgctgtggcgcacttgcaactggccgatggcgttttgaattaccagatcgatggcccggatgacgccccggtgctggtcctgtccaactcgctgggtaccgacctgggcatgtgggacacccagattccgctctggagtcagcacttccgggtgctgcgctatgacacccgtggtcacggcgcatcgctggtcactgaaggcccttacagcatcgaacagctgggccgcgacgtgctggccctgctcgatggcctggacattcaaaaggctcacttcgtcggcctgtcgatgggcggcctgatcggccagtggctgggtatccatgcaggtgagcgcctgcacagcctgaccctgtgcaacacggccgccaagatcgccaatgacgaggtgtggaacacccgtatcgacacggtactcaaaggcggccagcaggccatggtcgacctgcgcgatgcctccatcgcccgctggttcaccccgggctttgcccagggggatcctctagagtcgacctgcaggcatgcaagcttctagggataacagggtaatccggcgtaatcatggtcatagctgtttcctgtgtgaaattgttatccgctcacaattccacacaacatacgagccggaagcataaagtgtaaagcctggggtgcctaatgagtgagctaactcacattaattgcgttgcgctcactgcccgctttccagtcgggaaacctgtcgtgccagctgcattaatgaatcggccaacgcgcggggagaggcggtttgcgtattggggggtgggcgaagaactccagcatgagatccccgcgctggaggatcatccagccggcgtcccggaaaacgattccgaagcccaacctttcatagaaggcggcggtggaatcgaaatctcgtgatggcaggttgggcgtcgcttggtcggtcatttcgaaccccagagtcccgctcagaagaactcgtcaagaaggcgatagaaggcgatgcgctgcgaatcgggagcggcgataccgtaaagcacgaggaagcggtcagcccattcgccgccaagctcttcagcaatatcacgggtagccaacgctatgtcctgatagcggtccgccacacccagccggccacagtcgatgaatccagaaaagcggccattttccaccatgatattcggcaagcaggcatcgccatgggtcacgacgagatcctcgccgtcgggcatgcgcgccttgagcctggcgaacagttcggctggcgcgagcccctgatgctcttcgtccagatcatcctgatcgacaagaccggcttccatccgagtacgtgctcgctcgatgcgatgtttcgcttggtggtcgaatgggcaggtagccggatcaagcgtatgcagccgccgcattgcatcagccatgatggatactttctcggcaggagcaaggtgagatgacaggagatcctgccccggcacttcgcccaatagcagccagtcccttcccgcttcagtgacaacgtcgagcacagctgcgcaaggaacgcccgtcgtggccagccacgatagccgcgctgcctcgtcctgcagttcattcagggcaccggacaggtcggtcttgacaaaaagaaccgggcgcccctgcgctgacagccggaacacggcggcatcagagcagccgattgtctgttgtgcccagtcatagccgaatagcctctccacccaagcggccggagaacctgcgtgcaatccatcttgttcaatcatgcgaaacgatcctcatcctgtctcttgatcagatcttgatcccctgcgccatcagatccttggcggcaagaaagccatccagtttactttgcagggcttcccaaccttaccagagggcgccccagctggcaattccggttcgcttgctgtccataaaaccgcccagtctagctatcgccatgtaagcccactgcaagctacctgctttctctttgcgcttgcgttttcccttgtccagatagcccagtagctgacattcatccggggtcagcaccgtttctgcggactggctttctacgtgttccgcttcctttagcagcccttgcgccctgagtgcttgcggcagcgtgaagctaattcccatgtcagccgttaagtgttcctgtgtcactcaaaattgctttgagaggctctaagggcttctcagtgcgttacatccctggcttgttgtccacaaccgttaaaccttaaaagctttaaaagccttatatattcttttttttcttataaaacttaaaaccttagaggctatttaagttgctgatttatattaattttattgttcaaacatgagagcttagtacgtgaaacatgagagcttagtacgttagccatgagagcttagtacgttagccatgagggtttagttcgttaaacatgagagcttagtacgttaaacatgagagcttagtacgtgaaacatgagagcttagtacgtactatcaacaggttgaactgctgatcttcagatcctctacgccggacgcatcgtggccgttttccgctgcataaccctgcttcggggtcattatagcgattttttcggtatatccatcctttttcgcacgatatacaggattttgccaaagggttcgtgtagactttccttggtgtatccaacggcgtcagccgggcaggataggtgaagtaggcccacccgcgagcgggtgttccttcttcactgtcccttattcgcacctggcggtgctcaacgggaatcctgctctgcgaggctggccggctaccgccggcgtaacagatgagggcaagcggatggctgatgaaaccaagccaaccaggaagggcagcccacctatcaaggtgtactgccttccagacgaacgaagagcgattgaggaaaaggcggcggcggccggcatgagcctgtcggcctacctgctggccgtcggccagggctacaaaatcacgggcgtcgtggactatgagcacgtccgcgagctggcccgcatcaatggcgacctgggccgcctgggcggcctgctgaaactctggctcaccgacgacccgcgcacggcgcggttcggtgatgccacgatcctcgccctgctggcgaagatcgaagagaagcaggacgagcttggcaaggtcatgatgggcgtggtccgcccgagggcagagccatgacttttttagccgctaaaacggccggggggtgcgcgtgattgccaagcacgtccccatgcgctccatcaagaagagcgacttcgcggagctggtgaagtacatcaccgacgagcaaggcaagaccgaccaaagcggccatcgtgcctccccactcctgcagttcgggggcatggatgcgcggatagccgctgctggtttcctggatgccgacggatttgcactgccggtagaactccgcgaggtcgtccagcctcaggcagcagctgaaccaactcgcgaggggatcgagccccattcgccattcaggctgcgcaactgttgggaagggcgatcggtgcgggcctcttcgctattacgccagctggcgaaagggggatgtgctgcaaggcgattaagttgggtaacgccagggttttcccagtcacgacgttgtaaaacgacggccagtatagggataacagggtaatctgaattcgagctcggtaccc

SEQ ID NO: 55 - DNA, 4254 bp, artificial
  pEMG-pEM7
gccggcgtcccggaaaacgattccgaagcccaacctttcatagaaggcggcggtggaatcgaaatctcgtgatggcaggttgggcgtcgcttggtcggtcatttcgaaccccagagtcccgctcagaagaactcgtcaagaaggcgatagaaggcgatgcgctgcgaatcgggagcggcgataccgtaaagcacgaggaagcggtcagcccattcgccgccaagctcttcagcaatatcacgggtagccaacgctatgtcctgatagcggtccgccacacccagccggccacagtcgatgaatccagaaaagcggccattttccaccatgatattcggcaagcaggcatcgccatgggtcacgacgagatcctcgccgtcgggcatgcgcgccttgagcctggcgaacagttcggctggcgcgagcccctgatgctcttcgtccagatcatcctgatcgacaagaccggcttccatccgagtacgtgctcgctcgatgcgatgtttcgcttggtggtcgaatgggcaggtagccggatcaagcgtatgcagccgccgcattgcatcagccatgatggatactttctcggcaggagcaaggtgagatgacaggagatcctgccccggcacttcgcccaatagcagccagtcccttcccgcttcagtgacaacgtcgagcacagctgcgcaaggaacgcccgtcgtggccagccacgatagccgcgctgcctcgtcctgcagttcattcagggcaccggacaggtcggtcttgacaaaaagaaccgggcgcccctgcgctgacagccggaacacggcggcatcagagcagccgattgtctgttgtgcccagtcatagccgaatagcctctccacccaagcggccggagaacctgcgtgcaatccatcttgttcaatcatgcgaaacgatcctcatcctgtctcttgatcagatcttgatcccctgcgccatcagatccttggcggcaagaaagccatccagtttactttgcagggcttcccaaccttaccagagggcgccccagctggcaattccggttcgcttgctgtccataaaaccgcccagtctagctatcgccatgtaagcccactgcaagctacctgctttctctttgcgcttgcgttttcccttgtccagatagcccagtagctgacattcatccggggtcagcaccgtttctgcggactggctttctacgtgttccgcttcctttagcagcccttgcgccctgagtgcttgcggcagcgtgaagctaattcccatgtcagccgttaagtgttcctgtgtcactcaaaattgctttgagaggctctaagggcttctcagtgcgttacatccctggcttgttgtccacaaccgttaaaccttaaaagctttaaaagccttatatattcttttttttcttataaaacttaaaaccttagaggctatttaagttgctgatttatattaattttattgttcaaacatgagagcttagtacgtgaaacatgagagcttagtacgttagccatgagagcttagtacgttagccatgagggtttagttcgttaaacatgagagcttagtacgttaaacatgagagcttagtacgtgaaacatgagagcttagtacgtactatcaacaggttgaactgctgatcttcagatcctctacgccggacgcatcgtggccgttttccgctgcataaccctgcttcggggtcattatagcgattttttcggtatatccatcctttttcgcacgatatacaggattttgccaaagggttcgtgtagactttccttggtgtatccaacggcgtcagccgggcaggataggtgaagtaggcccacccgcgagcgggtgttccttcttcactgtcccttattcgcacctggcggtgctcaacgggaatcctgctctgcgaggctggccggctaccgccggcgtaacagatgagggcaagcggatggctgatgaaaccaagccaaccaggaagggcagcccacctatcaaggtgtactgccttccagacgaacgaagagcgattgaggaaaaggcggcggcggccggcatgagcctgtcggcctacctgctggccgtcggccagggctacaaaatcacgggcgtcgtggactatgagcacgtccgcgagctggcccgcatcaatggcgacctgggccgcctgggcggcctgctgaaactctggctcaccgacgacccgcgcacggcgcggttcggtgatgccacgatcctcgccctgctggcgaagatcgaagagaagcaggacgagcttggcaaggtcatgatgggcgtggtccgcccgagggcagagccatgacttttttagccgctaaaacggccggggggtgcgcgtgattgccaagcacgtccccatgcgctccatcaagaagagcgacttcgcggagctggtgaagtacatcaccgacgagcaaggcaagaccgaccaaagcggccatcgtgcctccccactcctgcagttcgggggcatggatgcgcggatagccgctgctggtttcctggatgccgacggatttgcactgccggtagaactccgcgaggtcgtccagcctcaggcagcagctgaaccaactcgcgaggggatcgagccccattcgccattcaggctgcgcaactgttgggaagggcgatcggtgcgggcctcttcgctattacgccagctggcgaaagggggatgtgctgcaaggcgattaagttgggtaacgccagggttttcccagtcacgacgttgtaaaacgacggccagtatagggataacagggtaatctgaattcgagctcggtaccctgggcgatgtgcagcagctcggcggcgcgggtgaagttcagggtctcggccaagactttgaagtaacgcaggtggcgcagctccatcagacctccagggtatggtgggagattcatttgatattggacggtcgtcagggtctcgcgcaatccttcagcaatcaagtaaacgcatcactcgggcctgcaactgaaagcccgacctgacgggacctggcaacacagctcaaggccgacgaaaaggaactggcccagcgcctgcagcgcgaaggcatctggcgtcacctgtggcgcattgccgggcattacgccaactacagcgtgttcgatgtgcccagcgtcgaggcattgcatgacacgctgatgcagctgccgctgttcccgtacatggatatcgaggtcgacggcctgtgtcggcatccctcgtctattcacagcgacgatcgctgattcgcacctgtatgcctgacaagaacaatacgaggtaagcacgttgttgacaattaatcatcggcatagtatatcggcatagtataatacgacaaggtgaggaactaaacccctaggttaaagaggagaaattaagcatgaccgtgaaaatttcccacactgccgacattcaagccttcttcaaccgggtagctggcctggaccatgccgaaggaaacccgcgcttcaagcagatcattctgcgcgtgctgcaagacaccgcccgcctgatcgaagacctggagattaccgaggacgagttctggcacgccgtcgactacctcaaccgcctgggcggccgtaacgaggcaggcctgctggctgctggcctgggtatcgagcacttcctcgacctgctgcaggatgccaaggatgccgaagccggccttggcggcggcaccccgcgcaccatcgaaggcccgttgtacgttgccggggcgccgctggcccagggcgaagcgcgcatggacgacggcactgacccaggcgtggtgatgttccttcagggccaggtgttcgatgccgacggcaagccgttggccggtgccaccgtcgacctgtggcacgccaatacccagggcacctattcgtacttcgaggggatcctctagagtcgacctgcaggcatgcaagcttctagggataacagggtaatccggcgtaatcatggtcatagctgtttcctgtgtgaaattgttatccgctcacaattccacacaacatacgagccggaagcataaagtgtaaagcctggggtgcctaatgagtgagctaactcacattaattgcgttgcgctcactgcccgctttccagtcgggaaacctgtcgtgccagctgcattaatgaatcggccaacgcgcggggagaggcggtttgcgtattggggggtgggcgaagaactccagcatgagatccccgcgctggaggatcatcca

SEQ ID NO: 56 - DNA, 40 bp, Artificial Sequence
  Primer sequence
caagcttaggaggaaaaacaaactggaagcggtgtcaaag

SEQ ID NO: 57 - DNA, 59 bp, Artificial Sequence
  Primer sequence
tcctcgcccttgctcaccatgcttaatttctcctctttgtggccggcattctatttgtc

SEQ ID NO: 58 - DNA, 21 bp, Artificial Sequence
  Primer sequence
aactggaagcggtgtcaaagc

SEQ ID NO: 59 - DNA, 19 bp, Artificial Sequence
  Primer sequence
gtggccggcattctatttg

SEQ ID NO: 60 - DNA, 40 bp, Artificial Sequence
  Primer sequence
caagcttaggaggaaaaacaccgcttcacagggaacacca

SEQ ID NO: 61 - DNA, 40 bp, Artificial Sequence
  Primer sequence
cctcgcccttgctcaccatcgatacaatcctccgcagaag

SEQ ID NO: 62 - DNA, 18 bp, Artificial Sequence
  Primer sequence
ccgcttcacagggaacac

SEQ ID NO: 63 - DNA, 21 bp, Artificial Sequence
  Primer sequence
cgatacaatcctccgcagaag

SEQ ID NO: 64 - DNA, 40 bp, Artificial Sequence
  Primer sequence
caagcttaggaggaaaaacagaaggaccggggccgcgcaa

SEQ ID NO: 65 - DNA, 40 bp, Artificial Sequence
  Primer sequence
tcctcgcccttgctcaccattgtcgatctctcccaaattg

SEQ ID NO: 66 - DNA, 40 bp, Artificial Sequence
  Primer sequence
tgaattcgagctcggtacccacaccgcgggcatgaccgcc

SEQ ID NO: 67 - DNA, 40 bp, Artificial Sequence
  Primer sequence
gtgcgccacagcggtctcctgcagcgtccttaatcatcat

SEQ ID NO: 68 - DNA, 40 bp, Artificial Sequence
  Primer sequence
atgatgattaaggacgctgcaggagaccgctgtggcgcac

SEQ ID NO: 69 - DNA, 40 bp, Artificial Sequence
  Primer sequence
gtcgactctagaggatccccctgggcaaagcccggggtga

SEQ ID NO: 70 - DNA, 45 bp, Artificial Sequence
  Primer sequence
taatctgaattcgagctcggtaccccgttggccggtgccaccgtc

SEQ ID NO: 71 - DNA, 50 bp, Artificial Sequence
  Primer sequence
gttcacggtcatgcttaatttctcctcttttcagccctcctgcaacgccc

SEQ ID NO: 72 - DNA, 20 bp, Artificial Sequence
  Primer sequence
gttcgaggttatgtcactgt

SEQ ID NO: 73 - DNA, 47 bp, Artificial Sequence
  Primer sequence
tgcaggtcgactctagaggatccccggcgggcagatcctgtgcgtag

SEQ ID NO: 74 - DNA, 45 bp, Artificial Sequence
  Primer sequence
gggctgaaaagaggagaaattaagcatgaccgtgaacatttccca

SEQ ID NO: 75 - DNA, 45 bp, Artificial Sequence
  Primer sequence
aaatcacagtgacataacctcgaactcaggcctcctgcaaagctc

SEQ ID NO: 76 - DNA, 45 bp, Artificial Sequence
  Primer sequence
taatctgaattcgagctcggtaccccgcgcctgaacgccgggcag

SEQ ID NO: 77 - DNA, 45 bp, Artificial Sequence
  Primer sequence
tctcccaccataccctggaggtctgacacaccatgcccacagggg

SEQ ID NO: 78 - DNA, 45 bp, Artificial Sequence
  Primer sequence
gccgcgagctttgcaggaggcctgatcatatggcctgttgctcga

SEQ ID NO: 79 - DNA, 45 bp, Artificial Sequence
  Primer sequence
tgcaggtcgactctagaggatcccctgaccaccttgcaacaggtg

SEQ ID NO: 80 - DNA, 20 bp, Artificial Sequence
  Primer sequence
cagacctccagggtatggtg

SEQ ID NO: 81 - DNA, 20 bp, Artificial Sequence
  Primer sequence
tcaggcctcctgcaaagctc

SEQ ID NO: 82 - DNA, 40 bp, Artificial Sequence
  Primer sequence
gtcgactctagaggatcccctcagccctcctgcaacgccc

SEQ ID NO: 83 - DNA, 20 bp, Artificial Sequence
  Primer sequence
atgaccgtgaaaatttccca

SEQ ID NO: 84 - DNA, 40 bp, Artificial Sequence
  Primer sequence
atatgtcgagctcggtacccgaaggaccggggccgcgcaa

SEQ ID NO: 85 - DNA, 40 bp, Artificial Sequence
  Primer sequence
tgggaaattttcacggtcattgtcgatctctcccaaattg

SEQ ID NO: 86 - DNA, 20 bp, Artificial Sequence
  Primer sequence
cgcgaattgcaagctgatcc

SEQ ID NO: 87 - DNA, 20 bp, Artificial Sequence
  Primer sequence
ctctcatccgccaaaacagc

SEQ ID NO: 88 - DNA, 501 bp, Artificial Sequence
  Promoter sequence
ccgcttcacagggaacaccactcaggcggtagggctgggagcggtaccaaagcagccaggtttcaggtttgattgaggaaacttgagaaaacgcttggcactaggacggcaggcaggtagaatgccggccacgcttggaggggtccccgagcggccaaaggggacgggctgtaaatccgttgcgagagcctcgaaggttcgagtcctcctccccccaccagttttagcgagggccgcaagccccgcgggtatagtttagtggtaaagcctcagccttccaagctgataatgcgggctcggttcccactacccgctccaagcttaccggatcttgcacagggtgtttcgctcttgtagcccagtcggtagaacacacccctggtaagggtgaggtcagcggctcaagtccgcttaaggactccgtatggacagggcgggtatgaaagtatctgcctctgttctgtcagtgcaagactaccccttctgcggaggattgtatcg

SEQ ID NO: 89 - DNA, 118 bp, Artificial Sequence
  Promoter sequence
aactggaagcggtgtcaaagcagctaagtttcagatttgattgaaaaaatttgaaaaaacgcttgacactaggacggcagacaaatagaatgccggccacaaagaggagaaattaagc

SEQ ID NO: 90 - DNA, 118 bp, Artificial Sequence
  Promoter sequence
aactggaagcggtgtcaaagcagctaggtttcggattcggttgacaaagtctggagggacgcttgacgttagggcggtagacaaatagaatgccggccacaaagaggagaaattaagc

SEQ ID NO: 91 - DNA, 116 bp, Artificial Sequence
  Promoter sequence
aactggaagcggtgtcaaagtagctgagttcggatctgattgaagaaatttgaaaaaacgcttggcactaggacggcagacaaatagaatgccggccacaaagaggagaaattaag

SEQ ID NO: 92 - DNA, 118 bp, Artificial Sequence
  Promoter sequence
aactggaagcggtgtcaaagtggctaggcttcagatttggttggaaaggtctgagaaaacgcttgacgctagagcggcagacaaatagaatgccggccacaaagaggagaaattaagc

SEQ ID NO: 93 - DNA, 119 bp, Artificial Sequence
  Promoter sequence
aactggaagcggtgtcaaagcagctgagcttcagatctgatcgagaagactcggggaaacgcttgacaccaggacagcagacaaatagaattgccggccacaaagaggagaaattaagc

SEQ ID NO: 94 - DNA, 118 bp, Artificial Sequence
  Promoter sequence
aactggaagcggtgtcaaagcagctgagtttcagacccgattggaaaggtttgaaggagcgcttgacactaggacggcagacaaatagaatgccggccacaaagaggagaaattaagc

SEQ ID NO: 95 - DNA, 118 bp, Artificial Sequence
  Promoter sequence
acctggaagcggtgtcaaagcagctgagtttcaggcctggttaagagagcttggaaaaacgtttgacactggggcggcagacaaatagaatgccggccacaaagaggagaaattaagc

SEQ ID NO: 96 - DNA, 118 bp, Artificial Sequence
  Promoter sequence
aactggaagcggtgtcaaagcagctaagtctcaggtttgattgggaaagtttggaaaagcgcttgacactaggacggcagacaaatagaatgccggccacaaagaggagaaattaagc

SEQ ID NO: 97 - DNA, 118 bp, Artificial Sequence
  Promoter sequence
aactggaagcggtgtcaaagcagctaaaccccaggtccggttgaagaagtttgaaaaaacgcttgacaccagggcggcagacaaatagaatgccggccacaaagaggagaaattaagc

SEQ ID NO: 98 - DNA, 118 bp, Artificial Sequence
  Promoter sequence
aactggaagcggtgtcaaagcagctaagtttcagacttgattgagaaaacttgaagaaacgcttgacaccaggatggcagacaaatagaatgccggccacaaagaggagaaattaagc

SEQ ID NO: 99 - DNA, 119 bp, Artificial Sequence
  Promoter sequence
aactggaagcggtgtcaaagcagctaagtttcagacttgattgaaagaatttggggaaacgcttgacactaggacggcagacaaatagaatgccggccacaaagaggagaaattaagct

SEQ ID NO: 100 - DNA, 118 bp, Artificial Sequence
  Promoter sequence
aactggaagcggtgtcaaagcagctaagtctcaggtttgatcgggaaagtctggaaaagcacttgacactagggcggcagacaaatagaatgccggccacaaagaggagaaattaagc

SEQ ID NO: 101 - DNA, 244 bp, Artificial Sequence
  Promoter sequence
gaaggaccggggccgcgcaagcggccccggtttttttttggcctgatgaaaaattttctatctcgagccttgtaatcggatgtggcggcctcatgtatgtggtcaccgcaaggtttctggtggcaacaccagacattacacaggtggttcgctcacagcgggccacccccggcaacgccggacagcatcaaaaccgccggtgtcgaaccggccgatgaaaaccacaatttgggagagatcgaca

SEQ ID NO: 102 - DNA, 244 bp, Artificial Sequence
  Promoter sequence
gaaggaccggggccgcgcaagcggccccggcttccctctggcctgatggagaatcctctaccccgagtcttgtggccgagtgcggcggcctcacgtatgtggtcaccgcagggcttctggtggtaacatcagatactgcacaggtggtccgctcacagcgggccacccccggcaacgccggacagcatcagaaccgccggtgccggaccggccgatgagagccacaatttgggagagatcgaca

SEQ ID NO: 103 - DNA, 244 bp, Artificial Sequence
  Promoter sequence
gaaggaccggggccgcgcaagtggctccggtttccctttggcccggtgaaaagtcttctaccttgagccctgtaatcggatgtggtagcctcatgtacgtggccaccgcgggatttctggtgacaacaccaggcatcacgcaggtggttcactcacagtgggccacccccggcaacgtcagacggcatcggaaccgccggtgtcgaaccggccgatgaaaaccacaatttgggagagatcgaca

SEQ ID NO: 104 - DNA, 244 bp, Artificial Sequence
  Promoter sequence
gaaggaccggggccgcgcaagtggctccggtttccctttggcccggtgaaaagtcttctaccttgagccctgtaatcggatgtggtagcctcatgtacgtggccaccgcgggatttctggtggcaacaccaggcatcacgcaggtggttcactcacagtgggccacccccggcaacgtcggacagcatcggaaccgccggtgtcgaaccggccgatgaaaaccgcaatttgggagagatcgaca

SEQ ID NO: 105 - DNA, 244 bp, Artificial Sequence
  Promoter sequence
gaaggaccggggccgcgcaagtggctccggtttccctttggcccggtgagaagtcttctaccttgagccctgtgatcggatgtggtagcctcatgtacgtggccaccgcgggatttctggtggcaacaccaggcatcacgcaggtggttcactcacagtgggccacccccggcaacgtcggacagcatcggaaccgccggtgtcgaaccggccgatgaaaaccacaatttgggagagatcgaca

SEQ ID NO: 106 - DNA, 4263 bp, Artificial Sequence
  Plasmid
ttaattaaagcggataacaatttcacacaggaggccgcctaggccgcggccgcgcgaattcgagctcggtacccggggatcctctagagtcgacctgcaggcatgcaagcttaggaggaaaaacatatggtgagcaagggcgaggaggataacatggccatcatcaaggagttcatgcgcttcaaggtgcacatggagggctccgtgaacggccacgagttcgagatcgagggcgagggcgagggccgcccctacgagggcacccagaccgccaagctgaaggtgaccaagggtggccccctgcccttcgcctgggacatcctgtcccctcagttcatgtacggctccaaggcctacgtgaagcaccccgccgacatccccgactacttgaagctgtccttccccgagggcttcaagtgggagcgcgtgatgaacttcgaggacggcggcgtggtgaccgtgacccaggactcctccctgcaagacggcgagttcatctacaaggtgaagctgcgcggcaccaacttcccctccgacggccccgtaatgcagaagaagaccatgggctgggaggcctcctccgagcggatgtaccccgaggacggcgccctgaagggcgagatcaagcagaggctgaagctgaaggacggcggccactacgacgctgaggtcaagaccacctacaaggccaagaagcccgtgcagctgcccggcgcctacaacgtcaacatcaagttggacatcacctcccacaacgaggactacaccatcgtggaacagtacgaacgcgccgagggccgccactccaccggcggcatggacgagctgtacaagtaaactagtcttggactcctgttgatagatccagtaatgacctcagaactccatctggatttgttcagaacgctcggttgccgccgggcgttttttattggtgagaatccaggggtccccaataattacgatttaaatttgtgtctcaaaatctctgatgttacattgcacaagataaaaatatatcatcatgaacaataaaactgtctgcttacataaacagtaatacaaggggtgttatgagccatattcagcgtgaaacgagctgtagccgtccgcgtctgaacagcaacatggatgcggatctgtatggctataaatgggcgcgtgataacgtgggtcagagcggcgcgaccatttatcgtctgtatggcaaaccggatgcgccggaactgtttctgaaacatggcaaaggcagcgtggcgaacgatgtgaccgatgaaatggtgcgtctgaactggctgaccgaatttatgccgctgccgaccattaaacattttattcgcaccccggatgatgcgtggctgctgaccaccgcgattccgggcaaaaccgcgtttcaggtgctggaagaatatccggatagcggcgaaaacattgtggatgcgctggccgtgtttctgcgtcgtctgcatagcattccggtgtgcaactgcccgtttaacagcgatcgtgtgtttcgtctggcccaggcgcagagccgtatgaacaacggcctggtggatgcgagcgattttgatgatgaacgtaacggctggccggtggaacaggtgtggaaagaaatgcataaactgctgccgtttagcccggatagcgtggtgacccacggcgattttagcctggataacctgattttcgatgaaggcaaactgattggctgcattgatgtgggccgtgtgggcattgcggatcgttatcaggatctggccattctgtggaactgcctgggcgaatttagcccgagcctgcaaaaacgtctgtttcagaaatatggcattgataatccggatatgaacaaactgcaatttcatctgatgctggatgaatttttctaataattaattggaccgcggtccgcgcgttgtccttttccgctgcataaccctgcttcggggtcattatagcgattttttcggtatatccatcctttttcgcacgatatacaggattttgccaaagggttcgtgtagactttccttggtgtatccaacggcgtcagccgggcaggataggtgaagtaggcccacccgcgagcgggtgttccttcttcactgtcccttattcgcacctggcggtgctcaacgggaatcctgctctgcgaggctggccgtaggccggccgataatctcatgaccaaaatcccttaacgtgagttttcgttccactgagcgtcagaccccgtagaaaagatcaaaggatcttcttgagatcctttttttctgcgcgtaatctgctgcttgcaaacaaaaaaaccaccgctaccagcggtggtttgtttgccggatcaagagctaccaactctttttccgaaggtaactggcttcagcagagcgcagataccaaatactgttcttctagtgtagccgtagttaggccaccacttcaagaactctgtagcaccgcctacatacctcgctctgctaatcctgttaccagtggctgctgccagtggcgataagtcgtgtcttaccgggttggactcaagacgatagttaccggataaggcgcagcggtcgggctgaacggggggttcgtgcacacagcccagcttggagcgaacgacctacaccgaactgagatacctacagcgtgagctatgagaaagcgccacgcttcccgaagggagaaaggcggacaggcatccggtaagcggcagggtcggaacaggagagcgcacgagggagcttccagggggaaacgcctggtatctttatagtcctgtcgggtttcgccacctctgacttgagcgtcgatttttgtgatgctcgtcaggggggcggagcctatggaaaaacgccagcaacgcggccgtgaaaggcaggccggtccgtggtggccacggcctctaggccagatccagcggcatctgggttagtcgagcgcgggccgcttcccatgtctcaccagggcgagcctgtttcgcgatctcagcatctgaaatcttcccggccttgcgcttcgctggggccttacccaccgccttggcgggcttcttcggtccaaaactgaacaacagatgtgtgaccttgcgcccggtctttcgctgcgcccactccacctgtagcgggctgtgctcgttgatctgcgtcacggctggatcaagcactcgcaacttgaagtccttgatcgagggataccggccttccagttgaaaccactttcgcagctggtcaatttctatttcgcgctggccgatgctgtcccattgcatgagcagctcgtaaagcctgatcgcgtgggtgctgtccatcttggccacgtcagccaaggcgtatttggtgaactgtttggtgagttccgtcaggtacggcagcatgtctttggtgaacctgagttctacacggccctcaccctcccggtagatgattgtttgcacccagccggtaatcatcacactcggtcttttccccttgccattgggctcttgggttaaccggacttcccgccgtttcaggcgcagggccgcttctttgagctggttgtaggaagattcgatagggacacccgccatcgtcgctatgtcctccgccgtcactgaatacatcacttcatcggtgacaggctcgctcctcttcacctggctaatacaggccagaacgatccgctgttcctgaacactgaggcgatacgcggcctcgaccagggcattgcttttgtaaaccattgggggtgaggccacgttcgacattccttgtgtataaggggacactgtatctgcgtcccacaatacaacaaatccgtccctttacaacaacaaatccgtcccttcttaacaacaaatccgtcccttaatggcaacaaatccgtccctttttaaactctacaggccacggattacgtggcctgtagacgtcctaaaaggtttaaaagggaaaaggaagaaaagggtggaaacgcaaaaaacgcaccactacgtggccccgttggggccgcatttgtgcccctgaaggggcgggggaggcgtctgggcaatccccgttttaccagtcccctatcgccgcctgagagggcgcaggaagcgagtaatcagggtatcgaggcggattcacccttggcgtccaaccagcggcaccagcggcgcctgagaggggcgcgcccagctgtctagggcggcggatttgtcctactcaggagagcgttcaccgacaaacaacagataaaacgaaaggcccagtctttcgactgagcctttcgttttatttgatgcct

SEQ ID NO: 107 - DNA, 5293 bp, Artificial Sequence
  Plasmid
tatgtcgagctcggtacccggggatcctctagagtcgacctgcaggcatgcaagcttggctgttttggcggatgagagaagattttcagcctgatacagattaaatcagaacgcagaagcggtctgataaaacagaatttgcctggcggcagtagcgcggtggtcccacctgaccccatgccgaactcagaagtgaaacgccgtagcgccgatggtagtgtggggtctccccatgcgagagtagggaactgccaggcatcaaataaaacgaaaggctcagtcgaaagactgggcctttcgttttatctgttgtttgtcggtgaacgctctcctgagtaggacaaatccgccgggagcggatttgaacgttgcgaagcaacggcccggagggtggcgggcaggacgcccgccataaactgccaggcatcaaattaagcagaaggccatcctgacggatggcctttttgcgtttctacaaactcttttgtttatttttctaaatacattcaaatatgtatccgctcatgagacaataaccctgataaatgcttcaataatattgaaaaaggaagagtatgagtattcaacatttccgtgtcgcccttattcccttttttgcggcattttgccttcctgtttttgctcacccagaaacgctggtgaaagtaaaagatgctgaagatcagttgggtgcacgagtgggttacatcgaactggatctcaacagcggtaagatccttgagagttttcgccccgaagaacgttttccaatgatgagcacttttaaagttctgctatgtggcgcggtattatcccgtgttgacgccgggcaagagcaactcggtcgccgcatacactattctcagaatgacttggttgagtactcaccagtcacagaaaagcatcttacggatggcatgacagtaagagaattatgcagtgctgccataaccatgagtgataacactgcggccaacttacttctgacaacgatcggaggaccgaaggagctaaccgcttttttgcacaacatgggggatcatgtaactcgccttgatcgttgggaaccggagctgaatgaagccataccaaacgacgagcgtgacaccacgatgcctgtagcaatggcaacaacgttgcgcaaactattaactggcgaactacttactctagcttcccggcaacaattaatagactggatggaggcggataaagttgcaggaccacttctgcgctcggcccttccggctggctggtttattgctgataaatctggagccggtgagcgtgggtctcgcggtatcattgcagcactggggccagatggtaagccctcccgtatcgtagttatctacacgacggggagtcaggcaactatggatgaacgaaatagacagatcgctgagataggtgcctcactgattaagcattggtaactgtcagaccaagtttactcatatatactttagattgatttaaaacttcatttttaatttaaaaggatctaggtgaagatcctttttgataatctcatgaccaaaatcccttaacgtgagttttcgttccactgagcgtcagaccccgtagaaaagatcaaaggatcttcttgagatcctttttttctgcgcgtaatctgctgcttgcaaacaaaaaaaccaccgctaccagcggtggtttgtttgccggatcaagagctaccaactctttttccgaaggtaactggcttcagcagagcgcagataccaaatactgtccttctagtgtagccgtagttaggccaccacttcaagaactctgtagcaccgcctacatacctcgctctgctaatcctgttaccagtggctgctgccagtggcgataagtcgtgtcttaccgggttggactcaagacgatagttaccggataaggcgcagcggtcgggctgaacggggggttcgtgcacacagcccagcttggagcgaacgacctacaccgaactgagatacctacagcgtgagctatgagaaagcgccacgcttcccgaagggagaaaggcggacaggtatccggtaagcggcagggtcggaacaggagagcgcacgagggagcttccagggggaaacgcctggtatctttatagtcctgtcgggtttcgccacctctgacttgagcgtcgatttttgtgatgctcgtcaggggggcggagcctatggaaaaacgccagcaacgcggcctttttacggttcctggccttttgctggccttttgctcacatgttctttcctgcgttatcccctgattctgtggataaccgtattaccgcctttgagtgagctgataccgctcgccgcagccgaacgaccgagcgcagcgagtcagtgagcgaggaagcggaagagcgcctgatgcggtattttctccttacgcatctgtgcggtatttcacaccgcatacggtgcactctcagtacaatctgctctgatgccgcatagttaagccagtatacactccgctatcgctacgtgactgggtcatggctgcgccccgacacccgccaacacccgctgacgcgccctgacgggcttgtctgctcccggcatccgcttacagacaagctgtgaccgtctccgggagctgcatgtgtcagaggttttcaccgtcatcaccgaaacgcgcgaggcagctgcggtaaagctcatcagcgtggtcgtgaagcgattcacagatgtctgcctgttcatccgcgtccagctcgttgagtttctccagaagcgttaatgtctggcttctgataaagcgggccatgttaagggcggttttttcctgtttggtcacttgatgcctccgtgtaagggggaatttctgttcatgggggtaatgataccgatgaaacgagagaggatgctcacgatacgggttactgatgatgaacatgcccggttactggaacgttgtgagggtaaacaactggcggtatggatgcggcgggaccagagaaaaatcactcagggtcaatgccagcgcttcgttaatacagatgtaggtgttccacagggtagccagcagcatcctgcgatgcagatccggaacataatggtgcagggcgctgacttccgcgtttccagactttacgaaacacggaaaccgaagaccattcatgttgttgctcaggtcgcagacgttttgcagcagcagtcgcttcacgttcgctcgcgtatcggtgattcattctgctaaccagtaaggcaaccccgccagcctagccgggtcctcaacgacaggagcacgatcatgcgcacccgtggccaggacccaacgctgcccgagatgcgccgcgtgcggctgctggagatggcggacgcgatggatatgttctgccaagggttggtttgcgcattcacagttctccgcaagaattgattggctccaattcttggagtggtgaatccgttagcgaggtgccgccggcttccattcaggtcgaggtggcccggctccatgcaccgcgacgcaacgcggggaggcagacaaggtatagggcggcgcctacaatccatgccaacccgttccatgtgctcgccgaggcggcataaatcgccgtgacgatcagcggtccagtgatcgaagttaggctggtaagagccgcgagcgatccttgaagctgtccctgatggtcgtcatctacctgcctggacagcatggcctgcaacgcgggcatcccgatgccgccggaagcgagaagaatcataatggggaaggccatccagcctcgcgtcgcgaacgccagcaagacgtagcccagcgcgtcggccagcttgcaattcgcgctaacttacattaattgcgttgcgctcactgcccgctttccagtcgggaaacctgtcgtgccagctgcattaatgaatcggccaacgcgcggggagaggcggtttgcgtattgggcgccagggtggtttttcttttcaccagtgagacgggcaacagctgattgcccttcaccgcctggccctgagagagttgcagcaagcggtccacgtggtttgccccagcaggcgaaaatcctgtttgatggtggttaacggcgggatataacatgagctgtcttcggtatcgtcgtatcccactaccgagatatccgcaccaacgcgcagcccggactcggtaatggcgcgcattgcgcccagcgccatctgatcgttggcaaccagcatcgcagtgggaacgatgccctcattcagcatttgcatggtttgttgaaaaccggacatggcactccagtcgccttcccgttccgctatcggctgaatttgattgcgagtgagatatttatgccagccagccagacgcagacgcgccgagacagaacttaatgggcccgctaacagcgcgatttgctggtgacccaatgcgaccagatgctccacgcccagtcgcgtaccgtcttcatgggagaaaataatactgttgatgggtgtctggtcagagacatcaagaaataacgccggaacattagtgcaggcagcttccacagcaatggcatcctggtcatccagcggatagttaatgatcagcccactgacgcgttgcgcgagaagattgtgcaccgccgctttacaggcttcgacgccgcttcgttctaccatcgacaccaccacgctggcacccagttgatcggcgcgagatttaatcgccgcgacaatttgcgacggcgcgtgcagggccagactggaggtggcaacgccaatcagcaacgactgtttgcccgccagttgttgtgccacgcggttgggaatgtaattcagctccgccatcgccgcttccactttttcccgcgttttcgcagaaacgtggctggcctggttcaccacgcgggaaacggtctgataagagacaccggcatactctgcgacatcgtataacgttactggtttcacattcaccaccctgaattgactctcttccgggcgctatcatgccataccgcgaaaggttttgcaccattcgatggtgtcaacgtaaatgccgcttcgccttcgcgcgcgaattgcaagctgatccgggcttatcgactgcacggtgcaccaatgcttctggcgtcaggcagccatcggaagctgtggtatggctgtgcaggtcgtaaatcactgcataattcgtgtcgctcaaggcgcactcccgttctggataatgttttttgcgccgacatcataacggttctggcaaatattctgaaatgagctgttgacaattaatcatcggctcgtataatgtgtggaattgtgagcggataacaatttcacacaggagatataca